European Patent Application EP 4 130 018 A1, published February 8, 2023. Title: METHOD FOR PRODUCING NUCLEIC ACID OLIGOMER. Applicant: SUMITOMO CHEMICAL COMPANY, LIMITED. The sequence listing filed with the application follows.

SEQUENCE LISTING (14 sequences)

SEQ ID NO: 1 - RNA, 21 nt, Artificial Sequence
  Synthetic oligonucleotide
  modified_base (7)..(7), (17)..(17): um
  modified_base (20)..(21): dT
auggaanacucuuggunacnn

SEQ ID NO: 2 - RNA, 21 nt, Artificial Sequence
  Synthetic oligonucleotide
  modified_base (2)..(2), (12)..(12), (14)..(15), (19)..(19): um
  modified_base (5)..(6), (16)..(17): cm
  modified_base (20)..(21): dT
gnaannaagagnannnnannn

SEQ ID NO: 3 - RNA, 36 nt, Artificial Sequence
  Synthetic oligonucleotide
agagccagccuucuuauuguuuuagagcuaugcugu

SEQ ID NO: 4 - RNA, 23 nt, Artificial Sequence
  Synthetic oligonucleotide
ccaugagaaguaugacaacagcc

SEQ ID NO: 5 - RNA, 25 nt, Artificial Sequence
  Synthetic oligonucleotide
ggcuguugucauacuucucaugguu

SEQ ID NO: 6 - RNA, 67 nt, Artificial Sequence
  Synthetic oligonucleotide
acagcauagcaaguuaaaauaaggcuaguccguuaucaacuugaaaaaguggcaccgagucggugcu

SEQ ID NO: 7 - RNA, 94 nt, Artificial Sequence
  Synthetic oligonucleotide
guuuucccuuuucaaagaaaucuccugggcaccuaucuucuuaggugcccucccuuguuuaaaccugaccaguuaaccggcugguuagguuuuu

SEQ ID NO: 8 - RNA, 100 nt, Artificial Sequence
  Synthetic oligonucleotide
aguccucaucucccucaagcguuuuagagcuaguaauagcaaguuaaaauaaggcuaguccguuaucaacuugaaaaaguggcaccgagucggugcuuuu

SEQ ID NO: 9 - RNA, 113 nt, Artificial Sequence
  Synthetic oligonucleotide
gcagauguaguguuuccacaguuuaagagcuaugcuggaaacagcauagcaaguuuaaauaaggcuaguccguuaucaacuugaaaaaguggcaccgagucggugcuuuuuuu

SEQ ID NO: 10 - RNA, 113 nt, Artificial Sequence
  Synthetic oligonucleotide
  modified_base (1)..(1), (8)..(8), (17)..(18): dA
  modified_base (2)..(2), (19)..(19): dG
  modified_base (3)..(3), (6)..(6), (9)..(9), (11)..(11), (15)..(15): dT
  modified_base (4)..(5), (7)..(7), (10)..(10), (12)..(14), (16)..(16), (20)..(20): dC
nnnnnnnnnnnnnnnnnnnnguuuaagagcuaugcugguaacagcauagcaaguuuaaauaaggcuaguccguuaucaacuugaaaaaguggcaccgagucggugcuuuuuuu

SEQ ID NO: 11 - RNA, 113 nt, Artificial Sequence
  Synthetic oligonucleotide
  modified_base (1)..(1): am
  modified_base (2)..(2): gm
  modified_base (3)..(3), (110)..(112): um
nnnccucaucucccucaagcguuuaagagcuaugcugguaacagcauagcaaguuuaaauaaggcuaguccguuaucaacuugaaaaaguggcaccgagucggugcuuunnnu

SEQ ID NO: 12 - RNA, 20 nt, Artificial Sequence
  Synthetic oligonucleotide
ggcaccgagucggugcuuuu

SEQ ID NO: 13 - RNA, 50 nt, Artificial Sequence
  Synthetic oligonucleotide
aaggcuaguccguuaucaacuugaaaaaguggcaccgagucggugcuuuu

SEQ ID NO: 14 - RNA, 100 nt, Artificial Sequence
  Synthetic oligonucleotide
auaacucaauuuguaaaaaaguuuuagagcuagaaauagcaaguuaaaauaaggcuaguccguuaucaacuugaaaaaguggcaccgagucggugcuuuu